European Patent Specification EP 3 865 574 B1, published July 19, 2023. Title: Variant of D-allulose 3-epimerase, manufacturing method thereof and manufacturing method of D-alluose using the same. Applicant: DAESANG CORPORATION. The sequence listing filed with the application follows.

SEQUENCE LISTING (12 sequences)

SEQ ID NO: 1 - protein, 294 aa, Unknown
  Wild type D-allulose 3-epimerase derived from Flavonifractor plautii
MNPIGMHYGFWSHNWDEIAYIPLMEKLAWLGFDICEVASAEWGYYDDARLRELKACADHNGLGITYSIGLEAKYDLASDDPAVRENGIRHVTRILESMPKVGAAILNGVSYAGWQALPDHGITLDEKRRKEELALESMSRLMKVAEDCGVLYCCEVVNRFEQYLLNTAKEGVEFVKRLGSPNARVLLDTFHMNIEEDSMVDAILEAGPWLGHFHVGENNRRPAGSTNRLPWKDMAAALKQVNYQGAIVMEPFVLMGGTIPYDIKVWRDLSGGAGEAGLDEMAGRACRFLKELTA

SEQ ID NO: 2 - protein, 294 aa, Artificial Sequence
  D-allulose 3-epimerase variant I21C
MNPIGMHYGFWSHNWDEIAYCPLMEKLAWLGFDICEVASAEWGYYDDARLRELKACADHNGLGITYSIGLEAKYDLASDDPAVRENGIRHVTRILESMPKVGAAILNGVSYAGWQALPDHGITLDEKRRKEELALESMSRLMKVAEDCGVLYCCEVVNRFEQYLLNTAKEGVEFVKRLGSPNARVLLDTFHMNIEEDSMVDAILEAGPWLGHFHVGENNRRPAGSTNRLPWKDMAAALKQVNYQGAIVMEPFVLMGGTIPYDIKVWRDLSGGAGEAGLDEMAGRACRFLKELTA

SEQ ID NO: 3 - protein, 294 aa, Artificial Sequence
  D-allulose 3-epimerase variant A82R
MNPIGMHYGFWSHNWDEIAYIPLMEKLAWLGFDICEVASAEWGYYDDARLRELKACADHNGLGITYSIGLEAKYDLASDDPRVRENGIRHVTRILESMPKVGAAILNGVSYAGWQALPDHGITLDEKRRKEELALESMSRLMKVAEDCGVLYCCEVVNRFEQYLLNTAKEGVEFVKRLGSPNARVLLDTFHMNIEEDSMVDAILEAGPWLGHFHVGENNRRPAGSTNRLPWKDMAAALKQVNYQGAIVMEPFVLMGGTIPYDIKVWRDLSGGAGEAGLDEMAGRACRFLKELTA

SEQ ID NO: 4 - protein, 294 aa, Artificial Sequence
  D-allulose 3-epimerase variant L133D
MNPIGMHYGFWSHNWDEIAYIPLMEKLAWLGFDICEVASAEWGYYDDARLRELKACADHNGLGITYSIGLEAKYDLASDDPAVRENGIRHVTRILESMPKVGAAILNGVSYAGWQALPDHGITLDEKRRKEEDALESMSRLMKVAEDCGVLYCCEVVNRFEQYLLNTAKEGVEFVKRLGSPNARVLLDTFHMNIEEDSMVDAILEAGPWLGHFHVGENNRRPAGSTNRLPWKDMAAALKQVNYQGAIVMEPFVLMGGTIPYDIKVWRDLSGGAGEAGLDEMAGRACRFLKELTA

SEQ ID NO: 5 - protein, 294 aa, Artificial Sequence
  D-allulose 3-epimerase variant G216S
MNPIGMHYGFWSHNWDEIAYIPLMEKLAWLGFDICEVASAEWGYYDDARLRELKACADHNGLGITYSIGLEAKYDLASDDPAVRENGIRHVTRILESMPKVGAAILNGVSYAGWQALPDHGITLDEKRRKEELALESMSRLMKVAEDCGVLYCCEVVNRFEQYLLNTAKEGVEFVKRLGSPNARVLLDTFHMNIEEDSMVDAILEAGPWLGHFHVSENNRRPAGSTNRLPWKDMAAALKQVNYQGAIVMEPFVLMGGTIPYDIKVWRDLSGGAGEAGLDEMAGRACRFLKELTA

SEQ ID NO: 6 - protein, 294 aa, Artificial Sequence
  D-allulose 3-epimerase variant A276R
MNPIGMHYGFWSHNWDEIAYIPLMEKLAWLGFDICEVASAEWGYYDDARLRELKACADHNGLGITYSIGLEAKYDLASDDPAVRENGIRHVTRILESMPKVGAAILNGVSYAGWQALPDHGITLDEKRRKEELALESMSRLMKVAEDCGVLYCCEVVNRFEQYLLNTAKEGVEFVKRLGSPNARVLLDTFHMNIEEDSMVDAILEAGPWLGHFHVGENNRRPAGSTNRLPWKDMAAALKQVNYQGAIVMEPFVLMGGTIPYDIKVWRDLSGGAGERGLDEMAGRACRFLKELTA

SEQ ID NO: 7 - DNA, 882 bp, Unknown
  Polynucleotide coding wild type D-allulose 3-epimerase derived from Flavonifractor plautii
atgaacccgattggaatgcactacggcttctggagccacaactgggacgagattgcatacatacccctgatggagaagctggcctggctgggctttgacatctgcgaggtggcctccgccgagtggggctattacgacgacgccaggctgcgggagctgaaggcctgcgccgatcacaacggcctgggcatcacctattccatcggcctggaggccaaatacgacctggccagcgacgatccggcggtgcgggagaacggcatccgccatgtcacccgcatcctggagagcatgcccaaggtgggggcggccatcctcaacggcgtgtcctacgccgggtggcaggccctgcccgaccacggaatcaccctggacgagaagcgccgcaaggaggagcttgccctggagtccatgtcccggctcatgaaggtggcggaggactgcggcgtgctctactgctgcgaggtggtcaaccgcttcgagcagtacctgctcaacaccgccaaagagggcgtggagtttgtcaagcgcctgggcagtcccaacgcccgggtgctgctggataccttccacatgaacatcgaggaggacagcatggtggacgccattctggaggcgggcccctggctggggcatttccacgtgggggagaacaaccgccgccccgccggctccaccaaccgcctgccctggaaggacatggccgccgccctcaagcaggtgaactaccagggggccattgtgatggagcccttcgtgctcatggggggtaccattccctatgatatcaaggtctggcgggatctcagcggcggggccggggaggccgggctggacgagatggcgggccgggcctgccggttcctcaaggagctgaccgcg

SEQ ID NO: 8 - DNA, 882 bp, Artificial Sequence
  Polynucleotide coding D-allulose 3-epimerase variant I21C
atgaacccgattggaatgcactacggcttctggagccacaactgggacgagattgcatactgccccctgatggagaagctggcctggctgggctttgacatctgcgaggtggcctccgccgagtggggctattacgacgacgccaggctgcgggagctgaaggcctgcgccgatcacaacggcctgggcatcacctattccatcggcctggaggccaaatacgacctggccagcgacgatccggcggtgcgggagaacggcatccgccatgtcacccgcatcctggagagcatgcccaaggtgggggcggccatcctcaacggcgtgtcctacgccgggtggcaggccctgcccgaccacggaatcaccctggacgagaagcgccgcaaggaggagcttgccctggagtccatgtcccggctcatgaaggtggcggaggactgcggcgtgctctactgctgcgaggtggtcaaccgcttcgagcagtacctgctcaacaccgccaaagagggcgtggagtttgtcaagcgcctgggcagtcccaacgcccgggtgctgctggataccttccacatgaacatcgaggaggacagcatggtggacgccattctggaggcgggcccctggctggggcatttccacgtgggggagaacaaccgccgccccgccggctccaccaaccgcctgccctggaaggacatggccgccgccctcaagcaggtgaactaccagggggccattgtgatggagcccttcgtgctcatggggggtaccattccctatgatatcaaggtctggcgggatctcagcggcggggccggggaggccgggctggacgagatggcgggccgggcctgccggttcctcaaggagctgaccgcg

SEQ ID NO: 9 - DNA, 882 bp, Artificial Sequence
  Polynucleotide coding D-allulose 3-epimerase variant A82R
atgaacccgattggaatgcactacggcttctggagccacaactgggacgagattgcatacatacccctgatggagaagctggcctggctgggctttgacatctgcgaggtggcctccgccgagtggggctattacgacgacgccaggctgcgggagctgaaggcctgcgccgatcacaacggcctgggcatcacctattccatcggcctggaggccaaatacgacctggccagcgacgatccgcgcgtgcgggagaacggcatccgccatgtcacccgcatcctggagagcatgcccaaggtgggggcggccatcctcaacggcgtgtcctacgccgggtggcaggccctgcccgaccacggaatcaccctggacgagaagcgccgcaaggaggagcttgccctggagtccatgtcccggctcatgaaggtggcggaggactgcggcgtgctctactgctgcgaggtggtcaaccgcttcgagcagtacctgctcaacaccgccaaagagggcgtggagtttgtcaagcgcctgggcagtcccaacgcccgggtgctgctggataccttccacatgaacatcgaggaggacagcatggtggacgccattctggaggcgggcccctggctggggcatttccacgtgggggagaacaaccgccgccccgccggctccaccaaccgcctgccctggaaggacatggccgccgccctcaagcaggtgaactaccagggggccattgtgatggagcccttcgtgctcatggggggtaccattccctatgatatcaaggtctggcgggatctcagcggcggggccggggaggccgggctggacgagatggcgggccgggcctgccggttcctcaaggagctgaccgcg

SEQ ID NO: 10 - DNA, 882 bp, Artificial Sequence
  Polynucleotide coding D-allulose 3-epimerase variant L133D
atgaacccgattggaatgcactacggcttctggagccacaactgggacgagattgcatacatacccctgatggagaagctggcctggctgggctttgacatctgcgaggtggcctccgccgagtggggctattacgacgacgccaggctgcgggagctgaaggcctgcgccgatcacaacggcctgggcatcacctattccatcggcctggaggccaaatacgacctggccagcgacgatccggcggtgcgggagaacggcatccgccatgtcacccgcatcctggagagcatgcccaaggtgggggcggccatcctcaacggcgtgtcctacgccgggtggcaggccctgcccgaccacggaatcaccctggacgagaagcgccgcaaggaggaggatgccctggagtccatgtcccggctcatgaaggtggcggaggactgcggcgtgctctactgctgcgaggtggtcaaccgcttcgagcagtacctgctcaacaccgccaaagagggcgtggagtttgtcaagcgcctgggcagtcccaacgcccgggtgctgctggataccttccacatgaacatcgaggaggacagcatggtggacgccattctggaggcgggcccctggctggggcatttccacgtgggggagaacaaccgccgccccgccggctccaccaaccgcctgccctggaaggacatggccgccgccctcaagcaggtgaactaccagggggccattgtgatggagcccttcgtgctcatggggggtaccattccctatgatatcaaggtctggcgggatctcagcggcggggccggggaggccgggctggacgagatggcgggccgggcctgccggttcctcaaggagctgaccgcg

SEQ ID NO: 11 - DNA, 882 bp, Artificial Sequence
  Polynucleotide coding D-allulose 3-epimerase variant G216S
atgaacccgattggaatgcactacggcttctggagccacaactgggacgagattgcatacatacccctgatggagaagctggcctggctgggctttgacatctgcgaggtggcctccgccgagtggggctattacgacgacgccaggctgcgggagctgaaggcctgcgccgatcacaacggcctgggcatcacctattccatcggcctggaggccaaatacgacctggccagcgacgatccggcggtgcgggagaacggcatccgccatgtcacccgcatcctggagagcatgcccaaggtgggggcggccatcctcaacggcgtgtcctacgccgggtggcaggccctgcccgaccacggaatcaccctggacgagaagcgccgcaaggaggagcttgccctggagtccatgtcccggctcatgaaggtggcggaggactgcggcgtgctctactgctgcgaggtggtcaaccgcttcgagcagtacctgctcaacaccgccaaagagggcgtggagtttgtcaagcgcctgggcagtcccaacgcccgggtgctgctggataccttccacatgaacatcgaggaggacagcatggtggacgccattctggaggcgggcccctggctggggcatttccacgtgagcgagaacaaccgccgccccgccggctccaccaaccgcctgccctggaaggacatggccgccgccctcaagcaggtgaactaccagggggccattgtgatggagcccttcgtgctcatggggggtaccattccctatgatatcaaggtctggcgggatctcagcggcggggccggggaggccgggctggacgagatggcgggccgggcctgccggttcctcaaggagctgaccgcg

SEQ ID NO: 12 - DNA, 882 bp, Artificial Sequence
  Polynucleotide coding D-allulose 3-epimerase variant A276R
atgaacccgattggaatgcactacggcttctggagccacaactgggacgagattgcatacatacccctgatggagaagctggcctggctgggctttgacatctgcgaggtggcctccgccgagtggggctattacgacgacgccaggctgcgggagctgaaggcctgcgccgatcacaacggcctgggcatcacctattccatcggcctggaggccaaatacgacctggccagcgacgatccggcggtgcgggagaacggcatccgccatgtcacccgcatcctggagagcatgcccaaggtgggggcggccatcctcaacggcgtgtcctacgccgggtggcaggccctgcccgaccacggaatcaccctggacgagaagcgccgcaaggaggagcttgccctggagtccatgtcccggctcatgaaggtggcggaggactgcggcgtgctctactgctgcgaggtggtcaaccgcttcgagcagtacctgctcaacaccgccaaagagggcgtggagtttgtcaagcgcctgggcagtcccaacgcccgggtgctgctggataccttccacatgaacatcgaggaggacagcatggtggacgccattctggaggcgggcccctggctggggcatttccacgtgggggagaacaaccgccgccccgccggctccaccaaccgcctgccctggaaggacatggccgccgccctcaagcaggtgaactaccagggggccattgtgatggagcccttcgtgctcatggggggtaccattccctatgatatcaaggtctggcgggatctcagcggcggggccggggagcgcgggctggacgagatggcgggccgggcctgccggttcctcaaggagctgaccgcg